European Patent Application EP 4 678 650 A1, published January 14, 2026. Title: METHOD FOR PREPARING POLYPEPTIDE SOLUTION FOR EVALUATING PHYSIOLOGICAL ACTIVITY AND METHOD FOR EVALUATING PHYSIOLOGICAL ACTIVITY OF POLYPEPTIDE. Applicant: FUJIFILM Corporation. The sequence listing filed with the application follows.

SEQUENCE LISTING (132 sequences)

SEQ ID NO: 1 - DNA, 123 bp, synthetic construct
  source 1..123: mol_type = other DNA
gttgtaaaacgacggccagtgccaagcttgggctaatacgactcactatagggagagtagttcaatggtagaacgtcggtctctaaaaccgagcgttgagggttcgattcctttctctcccac

SEQ ID NO: 2 - protein, 41 aa, synthetic construct
  MOD_RES 40: note = chloroacetylated lysine
  MOD_RES 19: note = chloroacetylated lysine
HCSYERLQFHGHEAPFRVKVSHCSYERLQFHGHEAPFRVKV

SEQ ID NO: 3 - protein, 6 aa, synthetic construct
VKKTKT

SEQ ID NO: 4 - protein, 11 aa, synthetic construct
VSGWRLFKKIS

SEQ ID NO: 5 - protein, 12 aa, synthetic construct
GVAMPGAEDDVV

SEQ ID NO: 6 - protein, 8 aa, synthetic construct
DYKDDDDK

SEQ ID NO: 7 - protein, 9 aa, synthetic construct
YPYDVPDYA

SEQ ID NO: 8 - protein, 6 aa, synthetic construct
HHHHHH

SEQ ID NO: 9 - protein, 10 aa, synthetic construct
EQKLISEEDL

SEQ ID NO: 10 - protein, 8 aa, synthetic construct
WSHPQFEK

SEQ ID NO: 11 - protein, 77 aa, synthetic construct
  MOD_RES 26: note = chloroacetylated lysine
  MOD_RES 47: note = chloroacetylated lysine
MVKKTKTHCSYERLQFHGHEAPFRVKVSHCSYERLQFHGHEAPFRVKVGSGVSGWRLFKKISSGSGVAMPGAEDDVV

SEQ ID NO: 12 - protein, 73 aa, synthetic construct
  MOD_RES 47: note = chloroacetylated lysine
  MOD_RES 26: note = chloroacetylated lysine
MVKKTKTHCSYERLQFHGHEAPFRVKVSHCSYERLQFHGHEAPFRVKVGSGVSGWRLFKKISSGSDYKDDDDK

SEQ ID NO: 13 - protein, 74 aa, synthetic construct
  MOD_RES 47: note = chloroacetylated lysine
  MOD_RES 26: note = chloroacetylated lysine
MVKKTKTHCSYERLQFHGHEAPFRVKVSHCSYERLQFHGHEAPFRVKVGSGVSGWRLFKKISSGSYPYDVPDYA

SEQ ID NO: 14 - protein, 71 aa, synthetic construct
  MOD_RES 26: note = chloroacetylated lysine
  MOD_RES 47: note = chloroacetylated lysine
MVKKTKTHCSYERLQFHGHEAPFRVKVSHCSYERLQFHGHEAPFRVKVGSGVSGWRLFKKISSGSHHHHHH

SEQ ID NO: 15 - protein, 75 aa, synthetic construct
  MOD_RES 26: note = chloroacetylated lysine
  MOD_RES 47: note = chloroacetylated lysine
MVKKTKTHCSYERLQFHGHEAPFRVKVSHCSYERLQFHGHEAPFRVKVGSGVSGWRLFKKISSGSEQKLISEEDL

SEQ ID NO: 16 - protein, 73 aa, synthetic construct
  MOD_RES 26: note = chloroacetylated lysine
  MOD_RES 47: note = chloroacetylated lysine
MVKKTKTHCSYERLQFHGHEAPFRVKVSHCSYERLQFHGHEAPFRVKVGSGVSGWRLFKKISSGSWSHPQFEK

SEQ ID NO: 17 - DNA, 322 bp, synthetic construct
  source 1..322: mol_type = other DNA
gaaattaatacgactcactatagggagaccacaacggtttccctctagaaataattttgtttaactttaagaaggagatataccaatggttaaaaaaacaaaaacacattgctcttacgaacgtctgcagttccatggtcatgaagctccgttccgtgtttaggtttcgcactgtagctatgagcgcttgcaatttcacggccacgaggcaccctttcgcgtataggtaggaagtggtgtaagtggatggcgattattcaagaagattagcagcggcagtggagttgcaatgcctggtgcagaagatgatgtagtataatga

SEQ ID NO: 18 - DNA, 310 bp, synthetic construct
  source 1..310: mol_type = other DNA
gaaattaatacgactcactatagggagaccacaacggtttccctctagaaataattttgtttaactttaagaaggagatataccaatggttaaaaaaacaaaaacacattgctcttacgaacgtctgcagttccatggtcatgaagctccgttccgtgtttaggtttcgcactgtagctatgagcgcttgcaatttcacggccacgaggcaccctttcgcgtataggtaggaagtggtgtaagtggatggcgattattcaagaagattagcagcggcagtgactacaaagacgacgacgacaaataatga

SEQ ID NO: 19 - DNA, 313 bp, synthetic construct
  source 1..313: mol_type = other DNA
gaaattaatacgactcactatagggagaccacaacggtttccctctagaaataattttgtttaactttaagaaggagatataccaatggttaaaaaaacaaaaacacattgctcttacgaacgtctgcagttccatggtcatgaagctccgttccgtgtttaggtttcgcactgtagctatgagcgcttgcaatttcacggccacgaggcaccctttcgcgtataggtaggaagtggtgtaagtggatggcgattattcaagaagattagcagcggcagttacccgtacgacgttccggactacgcttaatga

SEQ ID NO: 20 - DNA, 304 bp, synthetic construct
  source 1..304: mol_type = other DNA
gaaattaatacgactcactatagggagaccacaacggtttccctctagaaataattttgtttaactttaagaaggagatataccaatggttaaaaaaacaaaaacacattgctcttacgaacgtctgcagttccatggtcatgaagctccgttccgtgtttaggtttcgcactgtagctatgagcgcttgcaatttcacggccacgaggcaccctttcgcgtataggtaggaagtggtgtaagtggatggcgattattcaagaagattagcagcggcagtcatcatcatcatcatcattaatga

SEQ ID NO: 21 - DNA, 316 bp, synthetic construct
  source 1..316: mol_type = other DNA
gaaattaatacgactcactatagggagaccacaacggtttccctctagaaataattttgtttaactttaagaaggagatataccaatggttaaaaaaacaaaaacacattgctcttacgaacgtctgcagttccatggtcatgaagctccgttccgtgtttaggtttcgcactgtagctatgagcgcttgcaatttcacggccacgaggcaccctttcgcgtataggtaggaagtggtgtaagtggatggcgattattcaagaagattagcagcggcagtgaacagaaactgatctctgaagaagacctgtaatga

SEQ ID NO: 22 - DNA, 310 bp, synthetic construct
  source 1..310: mol_type = other DNA
gaaattaatacgactcactatagggagaccacaacggtttccctctagaaataattttgtttaactttaagaaggagatataccaatggttaaaaaaacaaaaacacattgctcttacgaacgtctgcagttccatggtcatgaagctccgttccgtgtttaggtttcgcactgtagctatgagcgcttgcaatttcacggccacgaggcaccctttcgcgtataggtaggaagtggtgtaagtggatggcgattattcaagaagattagcagcggcagttggtctcatccgcagttcgaaaaataatga

SEQ ID NO: 23 - DNA, 24 bp, synthetic construct
  source 1..24: mol_type = other DNA
gaaattaatacgactcactatagg

SEQ ID NO: 24 - DNA, 18 bp, synthetic construct
  source 1..18: mol_type = other DNA
cgaaacctaaacacggaa

SEQ ID NO: 25 - DNA, 105 bp, synthetic construct
  source 1..105: mol_type = other DNA
gaaattaatacgactcactatagggagaccacaacggtttccctctagaaataattttgtttaactttaagaaggagatataccaatggttaaaaaaacaaaaac

SEQ ID NO: 26 - DNA, 81 bp, synthetic construct
  source 1..81: mol_type = other DNA
cgaaacctaaacacggaacggagcttcatgaccatggaactgcagacgttcgtaagagcaatgtgtttttgtttttttaac

SEQ ID NO: 27 - DNA, 29 bp, synthetic construct
  source 1..29: mol_type = other DNA
tcattatactacatcatcttctgcaccag

SEQ ID NO: 28 - DNA, 19 bp, synthetic construct
  source 1..19: mol_type = other DNA
tcattatttgtcgtcgtcg

SEQ ID NO: 29 - DNA, 21 bp, synthetic construct
  source 1..21: mol_type = other DNA
tcattaagcgtagtccggaac

SEQ ID NO: 30 - DNA, 22 bp, synthetic construct
  source 1..22: mol_type = other DNA
tcattaatgatgatgatgatga

SEQ ID NO: 31 - DNA, 27 bp, synthetic construct
  source 1..27: mol_type = other DNA
tcattacaggtcttcttcagagatcag

SEQ ID NO: 32 - DNA, 20 bp, synthetic construct
  source 1..20: mol_type = other DNA
tcattatttttcgaactgcg

SEQ ID NO: 33 - DNA, 160 bp, synthetic construct
  source 1..160: mol_type = other DNA
catcatcttctgcaccaggcattgcaactccactgccgctgctaatcttcttgaataatcgccatccacttacaccacttcctacctatacgcgaaagggtgcctcgtggccgtgaaattgcaagcgctcatagctacagtgcgaaacctaaacacggaa

SEQ ID NO: 34 - DNA, 159 bp, synthetic construct
  source 1..159: mol_type = other DNA
tcattatttgtcgtcgtcgtctttgtagtcactgccgctgctaatcttcttgaataatcgccatccacttacaccacttcctacctatacgcgaaagggtgcctcgtggccgtgaaattgcaagcgctcatagctacagtgcgaaacctaaacacggaa

SEQ ID NO: 35 - DNA, 160 bp, synthetic construct
  source 1..160: mol_type = other DNA
attaagcgtagtccggaacgtcgtacgggtaactgccgctgctaatcttcttgaataatcgccatccacttacaccacttcctacctatacgcgaaagggtgcctcgtggccgtgaaattgcaagcgctcatagctacagtgcgaaacctaaacacggaa

SEQ ID NO: 36 - DNA, 153 bp, synthetic construct
  source 1..153: mol_type = other DNA
tcattaatgatgatgatgatgatgactgccgctgctaatcttcttgaataatcgccatccacttacaccacttcctacctatacgcgaaagggtgcctcgtggccgtgaaattgcaagcgctcatagctacagtgcgaaacctaaacacggaa

SEQ ID NO: 37 - DNA, 160 bp, synthetic construct
  source 1..160: mol_type = other DNA
acaggtcttcttcagagatcagtttctgttcactgccgctgctaatcttcttgaataatcgccatccacttacaccacttcctacctatacgcgaaagggtgcctcgtggccgtgaaattgcaagcgctcatagctacagtgcgaaacctaaacacggaa

SEQ ID NO: 38 - DNA, 159 bp, synthetic construct
  source 1..159: mol_type = other DNA
tcattatttttcgaactgcggatgagaccaactgccgctgctaatcttcttgaataatcgccatccacttacaccacttcctacctatacgcgaaagggtgcctcgtggccgtgaaattgcaagcgctcatagctacagtgcgaaacctaaacacggaa

SEQ ID NO: 39 - protein, 24 aa, synthetic construct
EQKLISEEDLGGSVSGWRLFKKIS

SEQ ID NO: 40 - protein, 10 aa, synthetic construct
  SITE 7..10: note = unsure
VKKTKTXXXX

SEQ ID NO: 41 - protein, 4 aa, synthetic construct
  REGION 1..4: note = VKKX Tag
VKKI

SEQ ID NO: 42 - protein, 4 aa, synthetic construct
  REGION 1..4: note = VKKX Tag
VKKK

SEQ ID NO: 43 - protein, 4 aa, synthetic construct
  REGION 1..4: note = VKKX Tag
VKKT

SEQ ID NO: 44 - protein, 4 aa, synthetic construct
  REGION 1..4: note = VKKX Tag
VKKR

SEQ ID NO: 45 - protein, 4 aa, synthetic construct
  REGION 1..4: note = VKKX Tag
VKKS

SEQ ID NO: 46 - protein, 4 aa, synthetic construct
  REGION 1..4: note = VKKX Tag
VKKH

SEQ ID NO: 47 - protein, 4 aa, synthetic construct
  REGION 1..4: note = VKKX Tag
VKKM

SEQ ID NO: 48 - protein, 4 aa, synthetic construct
  REGION 1..4: note = VKKX Tag
VKKP

SEQ ID NO: 49 - protein, 4 aa, synthetic construct
  REGION 1..4: note = VKKX Tag
VKKG

SEQ ID NO: 50 - protein, 4 aa, synthetic construct
  REGION 1..4: note = VKKX Tag
VKKL

SEQ ID NO: 51 - protein, 4 aa, synthetic construct
  REGION 1..4: note = VKKX Tag
VKKV

SEQ ID NO: 52 - protein, 4 aa, synthetic construct
  REGION 1..4: note = VKKX Tag
VKKE

SEQ ID NO: 53 - protein, 4 aa, synthetic construct
  REGION 1..4: note = VKKX Tag
VKKA

SEQ ID NO: 54 - protein, 4 aa, synthetic construct
  REGION 1..4: note = VKKX Tag
VKKD

SEQ ID NO: 55 - protein, 4 aa, synthetic construct
  REGION 1..4: note = VKKX Tag
VKKC

SEQ ID NO: 56 - protein, 4 aa, synthetic construct
  REGION 1..4: note = VKKX Tag
VKKN

SEQ ID NO: 57 - protein, 4 aa, synthetic construct
  REGION 1..4: note = VKKX Tag
VKKY

SEQ ID NO: 58 - protein, 4 aa, synthetic construct
  REGION 1..4: note = VKKX Tag
VKKQ

SEQ ID NO: 59 - protein, 4 aa, synthetic construct
  REGION 1..4: note = VKKX Tag
VKKW

SEQ ID NO: 60 - protein, 4 aa, synthetic construct
  REGION 1..4: note = VKKX Tag
VKKF

SEQ ID NO: 61 - protein, 6 aa, synthetic construct
  REGION 1..6: note = VKKX Tag
VKKTKT

SEQ ID NO: 62 - protein, 7 aa, synthetic construct
  REGION 1..7: note = VKKX Tag
VKKTKTT

SEQ ID NO: 63 - protein, 7 aa, synthetic construct
  REGION 1..7: note = VKKX Tag
VKKTKTD

SEQ ID NO: 64 - protein, 8 aa, synthetic construct
  REGION 1..8: note = VKKX Tag
VKKTKTKK

SEQ ID NO: 65 - protein, 8 aa, synthetic construct
  REGION 1..8: note = VKKX Tag
VKKTKTKT

SEQ ID NO: 66 - protein, 8 aa, synthetic construct
  REGION 1..8: note = VKKX Tag
VKKTKTKD

SEQ ID NO: 67 - protein, 8 aa, synthetic construct
  REGION 1..8: note = VKKX Tag
VKKTKTTK

SEQ ID NO: 68 - protein, 8 aa, synthetic construct
  REGION 1..8: note = VKKX Tag
VKKTKTTT

SEQ ID NO: 69 - protein, 8 aa, synthetic construct
  REGION 1..8: note = VKKX Tag
VKKTKTDD

SEQ ID NO: 70 - protein, 9 aa, synthetic construct
  REGION 1..9: note = VKKX Tag
VKKTKTKKT

SEQ ID NO: 71 - protein, 9 aa, synthetic construct
  REGION 1..9: note = VKKX Tag
VKKTKTKKD

SEQ ID NO: 72 - protein, 9 aa, synthetic construct
  REGION 1..9: note = VKKX Tag
VKKTKTKTK

SEQ ID NO: 73 - protein, 9 aa, synthetic construct
  REGION 1..9: note = VKKX Tag
VKKTKTKTT

SEQ ID NO: 74 - protein, 9 aa, synthetic construct
  REGION 1..9: note = VKKX Tag
VKKTKTKDK

SEQ ID NO: 75 - protein, 9 aa, synthetic construct
  REGION 1..9: note = VKKX Tag
VKKTKTKDT

SEQ ID NO: 76 - protein, 9 aa, synthetic construct
  REGION 1..9: note = VKKX Tag
VKKTKTKDD

SEQ ID NO: 77 - protein, 9 aa, synthetic construct
  REGION 1..9: note = VKKX Tag
VKKTKTTKK

SEQ ID NO: 78 - protein, 9 aa, synthetic construct
  REGION 1..9: note = VKKX Tag
VKKTKTTKT

SEQ ID NO: 79 - protein, 9 aa, synthetic construct
  REGION 1..9: note = VKKX Tag
VKKTKTTKD

SEQ ID NO: 80 - protein, 10 aa, synthetic construct
  REGION 1..10: note = VKKX Tag
VKKTKTKKTK

SEQ ID NO: 81 - protein, 10 aa, synthetic construct
  REGION 1..10: note = VKKX Tag
VKKTKTKKDK

SEQ ID NO: 82 - protein, 10 aa, synthetic construct
  REGION 1..10: note = VKKX Tag
VKKTKTKTKK

SEQ ID NO: 83 - protein, 10 aa, synthetic construct
  REGION 1..10: note = VKKX Tag
VKKTKTKTTK

SEQ ID NO: 84 - protein, 10 aa, synthetic construct
  REGION 1..10: note = VKKX Tag
VKKTKTKDKK

SEQ ID NO: 85 - protein, 10 aa, synthetic construct
  REGION 1..10: note = VKKX Tag
VKKTKTTTKK

SEQ ID NO: 86 - protein, 11 aa, synthetic construct
  REGION 1..11: note = VKKX Tag
VKKTKTKTDTT

SEQ ID NO: 87 - DNA, 12 bp, synthetic construct
  misc_feature 1..12: note = Code sequence of VKKX Tag
  source 1..12: mol_type = other DNA
gttaaaaaaata

SEQ ID NO: 88 - DNA, 12 bp, synthetic construct
  source 1..12: mol_type = other DNA
  misc_feature 1..12: note = Code sequence of VKKX Tag
gttaaaaaaaaa

SEQ ID NO: 89 - DNA, 12 bp, synthetic construct
  misc_feature 1..12: note = Code sequence of VKKX Tag
  source 1..12: mol_type = other DNA
gttaaaaaaaca

SEQ ID NO: 90 - DNA, 12 bp, synthetic construct
  misc_feature 1..12: note = Code sequence of VKKX Tag
  source 1..12: mol_type = other DNA
gttaaaaaacgg

SEQ ID NO: 91 - DNA, 12 bp, synthetic construct
  source 1..12: mol_type = other DNA
  misc_feature 1..12: note = Code sequence of VKKX Tag
gttaaaaaatca

SEQ ID NO: 92 - DNA, 12 bp, synthetic construct
  misc_feature 1..12: note = Code sequence of VKKX Tag
  source 1..12: mol_type = other DNA
gttaaaaaacat

SEQ ID NO: 93 - DNA, 12 bp, synthetic construct
  source 1..12: mol_type = other DNA
  misc_feature 1..12: note = Code sequence of VKKX Tag
gttaaaaaaatg

SEQ ID NO: 94 - DNA, 12 bp, synthetic construct
  source 1..12: mol_type = other DNA
  misc_feature 1..12: note = Code sequence of VKKX Tag
gttaaaaaacct

SEQ ID NO: 95 - DNA, 12 bp, synthetic construct
  misc_feature 1..12: note = Code sequence of VKKX Tag
  source 1..12: mol_type = other DNA
gttaaaaaaggc

SEQ ID NO: 96 - DNA, 12 bp, synthetic construct
  misc_feature 1..12: note = Code sequence of VKKX Tag
  source 1..12: mol_type = other DNA
gttaaaaaacta

SEQ ID NO: 97 - DNA, 12 bp, synthetic construct
  misc_feature 1..12: note = Code sequence of VKKX Tag
  source 1..12: mol_type = other DNA
gttaaaaaagtt

SEQ ID NO: 98 - DNA, 12 bp, synthetic construct
  misc_feature 1..12: note = Code sequence of VKKX Tag
  source 1..12: mol_type = other DNA
gttaaaaaagaa

SEQ ID NO: 99 - DNA, 12 bp, synthetic construct
  source 1..12: mol_type = other DNA
  misc_feature 1..12: note = Code sequence of VKKX Tag
gttaaaaaagca

SEQ ID NO: 100 - DNA, 12 bp, synthetic construct
  source 1..12: mol_type = other DNA
  misc_feature 1..12: note = Code sequence of VKKX Tag
gttaaaaaagat

SEQ ID NO: 101 - DNA, 12 bp, synthetic construct
  misc_feature 1..12: note = Code sequence of VKKX Tag
  source 1..12: mol_type = other DNA
gttaaaaaatgt

SEQ ID NO: 102 - DNA, 12 bp, synthetic construct
  source 1..12: mol_type = other DNA
  misc_feature 1..12: note = Code sequence of VKKX Tag
gttaaaaaaaat

SEQ ID NO: 103 - DNA, 12 bp, synthetic construct
  source 1..12: mol_type = other DNA
  misc_feature 1..12: note = Code sequence of VKKX Tag
gttaaaaaatat

SEQ ID NO: 104 - DNA, 12 bp, synthetic construct
  misc_feature 1..12: note = Code sequence of VKKX Tag
  source 1..12: mol_type = other DNA
gttaaaaaacaa

SEQ ID NO: 105 - DNA, 12 bp, synthetic construct
  source 1..12: mol_type = other DNA
  misc_feature 1..12: note = Code sequence of VKKX Tag
gttaaaaaatgg

SEQ ID NO: 106 - DNA, 12 bp, synthetic construct
  source 1..12: mol_type = other DNA
  misc_feature 1..12: note = Code sequence of VKKX Tag
gttaaaaaattt

SEQ ID NO: 107 - DNA, 18 bp, synthetic construct
  misc_feature 1..18: note = Code sequence of VKKX Tag
  source 1..18: mol_type = other DNA
gttaaaaaaacaaaaaca

SEQ ID NO: 108 - DNA, 21 bp, synthetic construct
  source 1..21: mol_type = other DNA
  misc_feature 1..21: note = Code sequence of VKKX Tag
gttaaaaaaacaaaaacaaca

SEQ ID NO: 109 - DNA, 21 bp, synthetic construct
  misc_feature 1..21: note = Code sequence of VKKX Tag
  source 1..21: mol_type = other DNA
gttaaaaaaacaaaaacagat

SEQ ID NO: 110 - DNA, 24 bp, synthetic construct
  misc_feature 1..24: note = Code sequence of VKKX Tag
  source 1..24: mol_type = other DNA
gttaaaaaaacaaaaacaaaaaaa

SEQ ID NO: 111 - DNA, 24 bp, synthetic construct
  source 1..24: mol_type = other DNA
  misc_feature 1..24: note = Code sequence of VKKX Tag
gttaaaaaaacaaaaacaaaaaca

SEQ ID NO: 112 - DNA, 24 bp, synthetic construct
  misc_feature 1..24: note = Code sequence of VKKX Tag
  source 1..24: mol_type = other DNA
gttaaaaaaacaaaaacaaaagat

SEQ ID NO: 113 - DNA, 24 bp, synthetic construct
  source 1..24: mol_type = other DNA
  misc_feature 1..24: note = Code sequence of VKKX Tag
gttaaaaaaacaaaaacaacaaaa

SEQ ID NO: 114 - DNA, 24 bp, synthetic construct
  source 1..24: mol_type = other DNA
  misc_feature 1..24: note = Code sequence of VKKX Tag
gttaaaaaaacaaaaacaacaaca

SEQ ID NO: 115 - DNA, 24 bp, synthetic construct
  misc_feature 1..24: note = Code sequence of VKKX Tag
  source 1..24: mol_type = other DNA
gttaaaaaaacaaaaacagatgat

SEQ ID NO: 116 - DNA, 27 bp, synthetic construct
  source 1..27: mol_type = other DNA
  misc_feature 1..27: note = Code sequence of VKKX Tage
gttaaaaaaacaaaaacaaaaaaaaca

SEQ ID NO: 117 - DNA, 27 bp, synthetic construct
  source 1..27: mol_type = other DNA
  misc_feature 1..27: note = Code sequence of VKKX Tag
gttaaaaaaacaaaaacaaaaaaagat

SEQ ID NO: 118 - DNA, 27 bp, synthetic construct
  source 1..27: mol_type = other DNA
  misc_feature 1..27: note = Code sequence of VKKX Tag
gttaaaaaaacaaaaacaaaaacaaaa

SEQ ID NO: 119 - DNA, 27 bp, synthetic construct
  misc_feature 1..27: note = Code sequence of VKKX Tag
  source 1..27: mol_type = other DNA
gttaaaaaaacaaaaacaaaaacaaca

SEQ ID NO: 120 - DNA, 27 bp, synthetic construct
  misc_feature 1..27: note = Code sequence of VKKX Tag
  source 1..27: mol_type = other DNA
gttaaaaaaacaaaaacaaaagataaa

SEQ ID NO: 121 - DNA, 27 bp, synthetic construct
  source 1..27: mol_type = other DNA
  misc_feature 1..27: note = Code sequence of VKKX Tag
gttaaaaaaacaaaaacaaaagataca

SEQ ID NO: 122 - DNA, 27 bp, synthetic construct
  misc_feature 1..27: note = Code sequence of VKKX Tag
  source 1..27: mol_type = other DNA
gttaaaaaaacaaaaacaaaagatgat

SEQ ID NO: 123 - DNA, 27 bp, synthetic construct
  misc_feature 1..27: note = Code sequence of VKKX Tag
  source 1..27: mol_type = other DNA
gttaaaaaaacaaaaacaacaaaaaaa

SEQ ID NO: 124 - DNA, 27 bp, synthetic construct
  misc_feature 1..27: note = Code sequence of VKKX Tag
  source 1..27: mol_type = other DNA
gttaaaaaaacaaaaacaacaaaaaca

SEQ ID NO: 125 - DNA, 27 bp, synthetic construct
  misc_feature 1..27: note = Code sequence of VKKX Tag
  source 1..27: mol_type = other DNA
gttaaaaaaacaaaaacaacaaaagat

SEQ ID NO: 126 - DNA, 30 bp, synthetic construct
  misc_feature 1..30: note = Code sequence of VKKX Tag
  source 1..30: mol_type = other DNA
gttaaaaaaacaaaaacaaaaaaaacaaaa

SEQ ID NO: 127 - DNA, 30 bp, synthetic construct
  misc_feature 1..30: note = Code sequence of VKKX Tag
  source 1..30: mol_type = other DNA
gttaaaaaaacaaaaacaaaaaaagataaa

SEQ ID NO: 128 - DNA, 30 bp, synthetic construct
  misc_feature 1..30: note = Code sequence of VKKX Tag
  source 1..30: mol_type = other DNA
gttaaaaaaacaaaaacaaaaacaaaaaaa

SEQ ID NO: 129 - DNA, 30 bp, synthetic construct
  misc_feature 1..30: note = Code sequence of VKKX Tag
  source 1..30: mol_type = other DNA
gttaaaaaaacaaaaacaaaaacaacaaaa

SEQ ID NO: 130 - DNA, 30 bp, synthetic construct
  source 1..30: mol_type = other DNA
  misc_feature 1..30: note = Code sequence of VKKX Tag
gttaaaaaaacaaaaacaaaagataaaaaa

SEQ ID NO: 131 - DNA, 30 bp, synthetic construct
  misc_feature 1..30: note = Code sequence of VKKX Tag
  source 1..30: mol_type = other DNA
gttaaaaaaacaaaaacaacaacaaaaaaa

SEQ ID NO: 132 - DNA, 33 bp, synthetic construct
  source 1..33: mol_type = other DNA
  misc_feature 1..33: note = Code sequence of VKKX Tag
gttaaaaaaacaaaaacaaaaacagatacaaca